European Patent Application EP 4 512 825 A9, published January 7, 2026. Title: 胶原蛋白及其用途. Applicant: 山西锦波生物医药股份有限公司. Application CN. The sequence listing filed with the application follows.

SEQUENCE LISTING (29 sequences)

SEQ ID NO: 1 - protein, 102 aa, synthetic construct
GKPGDDGEAGKPGKAGERGPPGPQGARGFPGTPGLPGVKGHRGYPGLDGAKGEAGAPGVKGESGSPGENGSPGPMGPRGLPGERGRTGPAGAAGARGNDGQP

SEQ ID NO: 2 - protein, 208 aa, synthetic construct
GKPGKAGERGPPGPQGARGFPGTPGLPGVKGHRGKPGKAGERGPPGPQGARGFPGTPGLPGVKGHRGKPGKAGERGPPGPQGARGFPGTPGLPGVKGHRGKPGKAGERGPPGPQGARGFPGTPGLPGVKGHRGKPGKAGERGPPGPQGARGFPGTPGLPGVKGHRGKPGKAGERGPPGPQGARGFPGTPGLPGVKGHRGKPGKAGERG

SEQ ID NO: 3 - protein, 168 aa, synthetic construct
GEPGREGSPGADGPPGRDGAAGVKGDRGETGAVGAPGAPGPPGSPGPAGPTGKQGDRGEAGAQGPMGPSGPAGARGIQGPQGPRGDKGEAGEPGERGLKGHRGFTGLQGLPGPPGPSGDQGASGPAGPSGPRGPPGPVGPSGKDGANGIPGPIGPPGPRGRSGETGPA

SEQ ID NO: 4 - protein, 90 aa, synthetic construct
GSPGPAGPTGKQGDRGEAGAQGPMGPSGPAGARGIQGPQGPRGDKGEAGEPGERGLKGHRGFTGLQGLPGPPGPSGDQGASGPAGPSGPR

SEQ ID NO: 5 - protein, 360 aa, synthetic construct
GARGIQGPQGPRGDKGEAGEPGERGLKGHRGFTGLQGLPGPPGPSGARGIQGPQGPRGDKGEAGEPGERGLKGHRGFTGLQGLPGPPGPSGARGIQGPQGPRGDKGEAGEPGERGLKGHRGFTGLQGLPGPPGPSGARGIQGPQGPRGDKGEAGEPGERGLKGHRGFTGLQGLPGPPGPSGARGIQGPQGPRGDKGEAGEPGERGLKGHRGFTGLQGLPGPPGPSGARGIQGPQGPRGDKGEAGEPGERGLKGHRGFTGLQGLPGPPGPSGARGIQGPQGPRGDKGEAGEPGERGLKGHRGFTGLQGLPGPPGPSGARGIQGPQGPRGDKGEAGEPGERGLKGHRGFTGLQGLPGPPGPS

SEQ ID NO: 6 - protein, 360 aa, synthetic construct
GSPGPAGPTGKQGDRGEAGAQGPMGPSGPAGARGIQGPQGPRGDKGEAGEPGERGLKGHRGFTGLQGLPGPPGPSGDQGASGPAGPSGPRGSPGPAGPTGKQGDRGEAGAQGPMGPSGPAGARGIQGPQGPRGDKGEAGEPGERGLKGHRGFTGLQGLPGPPGPSGDQGASGPAGPSGPRGSPGPAGPTGKQGDRGEAGAQGPMGPSGPAGARGIQGPQGPRGDKGEAGEPGERGLKGHRGFTGLQGLPGPPGPSGDQGASGPAGPSGPRGSPGPAGPTGKQGDRGEAGAQGPMGPSGPAGARGIQGPQGPRGDKGEAGEPGERGLKGHRGFTGLQGLPGPPGPSGDQGASGPAGPSGPR

SEQ ID NO: 7 - protein, 300 aa, synthetic construct
GPQGARGFPGTPGLPGVKGHRGYPGLDGAKGPQGARGFPGTPGLPGVKGHRGYPGLDGAKGPQGARGFPGTPGLPGVKGHRGYPGLDGAKGPQGARGFPGTPGLPGVKGHRGYPGLDGAKGPQGARGFPGTPGLPGVKGHRGYPGLDGAKGPQGARGFPGTPGLPGVKGHRGYPGLDGAKGPQGARGFPGTPGLPGVKGHRGYPGLDGAKGPQGARGFPGTPGLPGVKGHRGYPGLDGAKGPQGARGFPGTPGLPGVKGHRGYPGLDGAKGPQGARGFPGTPGLPGVKGHRGYPGLDGAK

SEQ ID NO: 8 - protein, 324 aa, synthetic construct
GARGFPGTPGLPGVKGHRGYPGLDGAKGARGFPGTPGLPGVKGHRGYPGLDGAKGARGFPGTPGLPGVKGHRGYPGLDGAKGARGFPGTPGLPGVKGHRGYPGLDGAKGARGFPGTPGLPGVKGHRGYPGLDGAKGARGFPGTPGLPGVKGHRGYPGLDGAKGARGFPGTPGLPGVKGHRGYPGLDGAKGARGFPGTPGLPGVKGHRGYPGLDGAKGARGFPGTPGLPGVKGHRGYPGLDGAKGARGFPGTPGLPGVKGHRGYPGLDGAKGARGFPGTPGLPGVKGHRGYPGLDGAKGARGFPGTPGLPGVKGHRGYPGLDGAK

SEQ ID NO: 9 - protein, 336 aa, synthetic construct
GFPGTPGLPGVKGHRGYPGLDGAKGFPGTPGLPGVKGHRGYPGLDGAKGFPGTPGLPGVKGHRGYPGLDGAKGFPGTPGLPGVKGHRGYPGLDGAKGFPGTPGLPGVKGHRGYPGLDGAKGFPGTPGLPGVKGHRGYPGLDGAKGFPGTPGLPGVKGHRGYPGLDGAKGFPGTPGLPGVKGHRGYPGLDGAKGFPGTPGLPGVKGHRGYPGLDGAKGFPGTPGLPGVKGHRGYPGLDGAKGFPGTPGLPGVKGHRGYPGLDGAKGFPGTPGLPGVKGHRGYPGLDGAKGFPGTPGLPGVKGHRGYPGLDGAKGFPGTPGLPGVKGHRGYPGLDGAK

SEQ ID NO: 10 - protein, 336 aa, synthetic construct
GTPGLPGVKGHRGYPGLDGAKGTPGLPGVKGHRGYPGLDGAKGTPGLPGVKGHRGYPGLDGAKGTPGLPGVKGHRGYPGLDGAKGTPGLPGVKGHRGYPGLDGAKGTPGLPGVKGHRGYPGLDGAKGTPGLPGVKGHRGYPGLDGAKGTPGLPGVKGHRGYPGLDGAKGTPGLPGVKGHRGYPGLDGAKGTPGLPGVKGHRGYPGLDGAKGTPGLPGVKGHRGYPGLDGAKGTPGLPGVKGHRGYPGLDGAKGTPGLPGVKGHRGYPGLDGAKGTPGLPGVKGHRGYPGLDGAKGTPGLPGVKGHRGYPGLDGAKGTPGLPGVKGHRGYPGLDGAK

SEQ ID NO: 11 - protein, 312 aa, synthetic construct
GERGLKGHRGFTGLQGLPGPPGPSGDQGASGPAGPSGPRGERGLKGHRGFTGLQGLPGPPGPSGDQGASGPAGPSGPRGERGLKGHRGFTGLQGLPGPPGPSGDQGASGPAGPSGPRGERGLKGHRGFTGLQGLPGPPGPSGDQGASGPAGPSGPRGERGLKGHRGFTGLQGLPGPPGPSGDQGASGPAGPSGPRGERGLKGHRGFTGLQGLPGPPGPSGDQGASGPAGPSGPRGERGLKGHRGFTGLQGLPGPPGPSGDQGASGPAGPSGPRGERGLKGHRGFTGLQGLPGPPGPSGDQGASGPAGPSGPR

SEQ ID NO: 12 - protein, 330 aa, synthetic construct
GERGLKGHRGFTGLQGLPGPPGPSGDQGASGPAGERGLKGHRGFTGLQGLPGPPGPSGDQGASGPAGERGLKGHRGFTGLQGLPGPPGPSGDQGASGPAGERGLKGHRGFTGLQGLPGPPGPSGDQGASGPAGERGLKGHRGFTGLQGLPGPPGPSGDQGASGPAGERGLKGHRGFTGLQGLPGPPGPSGDQGASGPAGERGLKGHRGFTGLQGLPGPPGPSGDQGASGPAGERGLKGHRGFTGLQGLPGPPGPSGDQGASGPAGERGLKGHRGFTGLQGLPGPPGPSGDQGASGPAGERGLKGHRGFTGLQGLPGPPGPSGDQGASGPA

SEQ ID NO: 13 - protein, 324 aa, synthetic construct
GERGLKGHRGFTGLQGLPGPPGPSGDQGERGLKGHRGFTGLQGLPGPPGPSGDQGERGLKGHRGFTGLQGLPGPPGPSGDQGERGLKGHRGFTGLQGLPGPPGPSGDQGERGLKGHRGFTGLQGLPGPPGPSGDQGERGLKGHRGFTGLQGLPGPPGPSGDQGERGLKGHRGFTGLQGLPGPPGPSGDQGERGLKGHRGFTGLQGLPGPPGPSGDQGERGLKGHRGFTGLQGLPGPPGPSGDQGERGLKGHRGFTGLQGLPGPPGPSGDQGERGLKGHRGFTGLQGLPGPPGPSGDQGERGLKGHRGFTGLQGLPGPPGPSGDQ

SEQ ID NO: 14 - protein, 336 aa, synthetic construct
GERGLKGHRGFTGLQGLPGPPGERGLKGHRGFTGLQGLPGPPGERGLKGHRGFTGLQGLPGPPGERGLKGHRGFTGLQGLPGPPGERGLKGHRGFTGLQGLPGPPGERGLKGHRGFTGLQGLPGPPGERGLKGHRGFTGLQGLPGPPGERGLKGHRGFTGLQGLPGPPGERGLKGHRGFTGLQGLPGPPGERGLKGHRGFTGLQGLPGPPGERGLKGHRGFTGLQGLPGPPGERGLKGHRGFTGLQGLPGPPGERGLKGHRGFTGLQGLPGPPGERGLKGHRGFTGLQGLPGPPGERGLKGHRGFTGLQGLPGPPGERGLKGHRGFTGLQGLPGPP

SEQ ID NO: 15 - protein, 42 aa, Homo sapiens
GTPGLPGVKGHRGYPGLDGAKGTPGLPGVKGHRGYPGLDGAK

SEQ ID NO: 16 - DNA, 306 bp, synthetic construct
  source 1..306: mol_type = other DNA
ggtaaaccaggagatgatggagaagcaggaaaaccaggaaaagcaggagaaagaggaccgcctggaccgcaaggagcacgtggatttccaggaaccccgggactgccgggtgtgaaaggtcatagaggatatccgggactggatggagcaaaaggagaagcaggggcaccgggagttaaaggtgagagcggaagcccgggagaaaatggaagccctggtccgatgggtccgagagggctgccgggtgaaagagggcgtaccggtccggcaggagcagcaggtgcaagaggaaatgatggacagccg

SEQ ID NO: 17 - DNA, 623 bp, synthetic construct
  source 1..623: mol_type = other DNA
ggaaaacccgggaaggccggtgagcgcggtccaccgggtccgcagggcgcgcgtgggttcccgggcaccccgggtctgccgggtgttaaaggtcatcgtggcaagccgggcaaggctggcgagcgcggtccgccaggtccgcaaggtgcgagaggctttccgggcactccgggtttgccgggtgtcaaaggtcaccgtggtaaaccgggcaaggcgggtgagcgtggcccaccgggtccgcagggtgcgcgtggttttccgggcacgccgggtttgccgggcgttaaaggccaccgcggcaaaccgggcaaggcgggtgaacgtggcccaccgggtccgcaaggtgcacgtggcttcccgggcaccccgggtctgcctggcgtgaaaggtcaccgtggcaagccgggcaaagctggtgaacgtggtccgcccggtccgcagggcgcgcgtggctttccgggaaccccgggcctgccgggcgttaagggtcatcgtggcaaaccgggcaaggctggtgagcgcgggccaccgggtcctcaaggtgcccgtggcttcccgggcaccccgggtctgccgggtgtgaagggtcaccgcggtaaaccgggcaaggcaggcgaacgcgg

SEQ ID NO: 18 - DNA, 503 bp, synthetic construct
  source 1..503: mol_type = other DNA
gtgaaccaggtcgtgaaggtagcccaggtgcagatggaccaccaggtcgtgatggtgcagcaggagtgaaaggagatcgtggtgaaaccggtgcagtaggtgcacctggtgcgccaggtccgccaggtagccctggtccagccggtcctaccggaaaacaaggggatagaggagaagcaggagcacagggtccgatgggtccgtcaggtccggcgggtgcacgtggtattcagggtccgcagggtccgcgtggtgataaaggtgaagcaggtgaaccgggggaaagaggattaaaagggcatcgtggttttacgggtctgcagggtctgcctggtccgcctggtccgagcggtgatcagggtgcaagcggtccggcaggtccgagcggacctcgtggacctccgggtcctgtgggtcctagtggtaaggatggggcaaatggtattcctggtcctattggtccgccgggtccgcgtgggagatcaggtgaaaccggaccggca

SEQ ID NO: 19 - DNA, 270 bp, synthetic construct
  source 1..270: mol_type = other DNA
ggtagcccaggtccagcaggtccgacaggtaaacaaggagatcgtggtgaagcaggagcacaaggaccaatgggtccaagcggtccggcaggtgcaagaggtattcaagggccgcaagggccacgcggtgataaaggggaagcaggtgaaccaggtgagagagggttaaaaggacatcgtggatttacaggactgcagggtttaccaggtccgccgggaccgagcggagatcaaggtgcaagcggtccggcgggtccgagtggtcctcgt

SEQ ID NO: 20 - DNA, 1080 bp, synthetic construct
  source 1..1080: mol_type = other DNA
ggagctaggggtatccagggtccgcagggcccgcggggagataaaggggaagcgggtgaaccgggtgaacgtggcttgaagggtcatcgtggcttcaccggcctgcagggcttgccgggtccgccgggtccgtccggtgcccgtggcatccagggaccgcaaggaccgcgtggagacaaaggtgaagcgggtgaaccgggtgagcgcggcctcaagggccaccgcggcttcaccggtttgcaaggcctgccgggtccgccgggtccgtcgggcgcgcgtggtattcaaggcccgcaaggtccacgcggcgacaaaggcgaagcgggtgagccgggcgaacgcggcctgaaaggtcaccgcggttttacgggtctgcagggcctgccgggtccaccgggtccgagcggtgctcgcggcatccagggcccgcaaggtccgcgtggtgataagggtgaggcgggtgagccgggagaacgtggtctgaagggtcatagaggcttcaccggtctgcaaggtctgccgggtccaccgggcccgagcggcgctaggggcattcagggcccgcaggggccgcgtggtgataagggcgaggccggtgagccgggcgaacgtggtttaaaaggtcatcgcggcttcacgggcctccaaggtctgcctggcccaccgggtccgagcggcgcgcgtggcattcaaggcccacagggtcctcgtggcgacaaaggcgaggcaggcgagccgggtgagcgcggtctgaaagggcaccgtggttttaccggtttgcaaggcctgccgggcccaccgggcccgtccggtgcacgtggcattcagggtccgcagggtccgcgtggcgacaagggcgaagctggtgagccgggtgagcgcggccttaagggtcaccgtggctttaccggtttacaaggtttgccgggccctccgggtccaagcggtgcacgtggtatccaaggcccacagggtccgcgtggggataaaggcgaagcgggtgaaccgggcgagcgcgggctgaagggtcaccgtggctttactggcctgcagggtctgccgggtccaccgggtccgtct

SEQ ID NO: 21 - DNA, 1083 bp, synthetic construct
  source 1..1083: mol_type = other DNA
ggatcacccgggccggcgggcccgaccggtaaacagggtgaccgcggtgaggcgggtgcgcaggggccgatgggtccgagcggtccggctggtgcgcgtggtatccagggaccgcagggcccacgcggtgataaaggcgaagcaggcgaaccgggtgagcgcggtttgaagggccaccgtggttttaccggtctgcagggcctgccgggcccgccgggtccgtcaggcgatcagggtgctagcggtccggctggcccgtccggcccgcgcggtagcccgggcccagctggcccgactggtaaacagggcgaccgtggcgaggccggtgcccaaggccctatgggcccgagcggtccggcaggcgcgcggggcatccagggtccgcaaggaccaagaggcgacaagggtgaggcaggcgagcctggcgaacgtggcctgaagggtcaccgcggttttaccggtctccaaggtctgcctggtccaccgggtccgtctggagatcaaggcgccagcggccccgcgggtccctccggtccgcgtggcagcccgggtccggcaggaccaacgggtaagcagggtgatagaggcgaagccggtgcgcagggcccgatgggtccttcgggtccagcgggggcgcgtggcattcaaggtccgcagggcccgcgtggtgacaaaggtgaggcgggcgaaccgggcgagcgcggcttgaagggtcatcgtggattcaccggtttgcaaggcctgccgggccccccgggcccgagcggtgaccaaggagctagcgggccggctggtccgtcgggcccgcgtggcagtccgggtccggcgggcccaacgggcaagcaaggagatcgtggtgaggcgggtgcgcaaggtccgatgggtccgtctggtccggcgggtgcacgcggtattcaaggtccgcaggggccgcgtggtgataaaggagaagcaggcgaaccgggtgaacgtggtctgaaaggtcatcgtggcttcaccggcctgcagggtttaccaggtccaccgggtccgtctggcgaccagggtgccagcggtccggcgggcccgtccggaccgcgttaa

SEQ ID NO: 22 - DNA, 900 bp, synthetic construct
  source 1..900: mol_type = other DNA
ggaccccaaggggcgcgtggttttccgggcaccccgggcctgccgggcgtgaagggtcaccgcggttatccggggctggatggcgcgaagggtccgcaaggtgctcgcggtttcccgggaaccccgggcctgccgggcgttaaaggtcatcgtggttatccgggtctggatggtgcgaagggcccacagggtgcgcgtggtttcccgggcacccctgggctcccgggtgtgaaaggtcacagaggttacccgggcctggatggtgccaaaggtccgcaaggtgcgcgtggttttccgggcacgccgggcttgccgggtgttaaaggtcaccgtggttatccgggtctggacggcgcaaagggtcctcagggtgcacgcggcttcccgggtacgccgggccttccgggcgtgaagggccaccgcggttatccgggtttggacggtgccaagggtccgcagggtgcgcgtggattcccgggaaccccaggcctgccaggtgtgaagggccaccgtggctacccgggcttggacggtgctaaaggaccgcagggcgcacgtggctttccgggtaccccgggcctgcctggcgtcaagggccatcgtggttacccgggcctggatggtgcaaaaggcccacagggtgcccgtggtttcccgggtactccgggcctgccgggcgtaaaaggccatcgcggttacccgggtttggatggcgctaaaggcccacaaggtgctagagggttccctggcaccccgggtctgccgggcgttaaaggccatcgtggttacccgggcttggacggcgcgaagggtccgcaaggcgcgcgtggttttccgggtaccccgggtctgccaggcgttaagggtcaccgcggttacccgggtttagacggtgcgaaa

SEQ ID NO: 23 - DNA, 972 bp, synthetic construct
  source 1..972: mol_type = other DNA
ggtgctaggggattcccgggaaccccgggtctgccaggcgtgaaaggtcaccgcggttacccgggcctcgacggcgcgaagggtgcccgtggttttccgggaaccccgggcttgccaggtgtcaagggccatcgtggttacccgggtctcgatggtgcaaagggtgcgagaggcttcccgggcaccccgggcctgccaggggtgaaaggccacagaggctatcctggcttggatggtgccaagggtgcacgtggattcccgggcactccgggtctgccgggcgtgaagggccaccgcggttatccgggcctggacggtgctaaaggcgcgcgtggttttccgggtacgccgggcttgccaggtgttaagggccaccgtggctacccggggctggatggtgccaaaggtgctcgcggtttcccgggaaccccgggtctgcctggcgtgaagggtcatcgtggttacccgggcttggacggcgctaagggtgcgcgtggttttccgggcaccccgggtctgccgggggtgaaaggtcaccgcggttatcccggtctggatggtgcgaagggtgcgcgtggcttcccgggcaccccgggcctgccgggtgttaaaggtcatcgtggttacccgggcctggatggtgccaagggcgctcgcggttttccgggcacgccaggtttaccgggggtcaaaggccatcgtggctatccgggtttagatggcgcgaaaggcgcacgcggattcccgggaaccccgggcctgcctggcgttaaaggccaccgcggttacccgggccttgacggcgcgaaaggcgcgcgtggttttccgggcaccccgggtctgccgggtgttaaaggtcaccgtggctatccgggtctggacggtgcaaaaggtgcacgtggtttcccggggactccgggcctgccgggtgttaagggccatcgtggttacccgggtttggacggtgcgaag

SEQ ID NO: 24 - DNA, 1008 bp, synthetic construct
  source 1..1008: mol_type = other DNA
ggatttcccgggactccaggtctgcccggcgtgaagggccaccgcggttatccgggcttggacggtgcgaaaggcttcccgggcacgccaggcttacctggtgtgaagggccatcgtggttacccggggctggatggtgcgaagggttttccgggcaccccgggtctgccgggcgtaaagggccaccgcggttatccgggcctggacggtgcaaaaggttttccgggcaccccgggcctgccgggtgtgaagggccaccgcggttacccgggtttggacggtgccaagggattcccaggtacgccgggtctgccgggggtgaagggccatagaggctacccgggcttggatggtgcgaaaggtttcccgggaacccctggtctgccgggcgttaagggccaccgtggttatccgggtctggatggcgcgaaaggttttccgggaaccccaggtctgccgggcgttaaaggtcatcgtggttacccggggctcgatggtgccaaaggttttccgggcaccccgggtctgccgggcgtcaaaggtcaccgcggttatccgggtctggatggtgcgaaaggcttcccgggaaccccgggcctgcctggcgtgaaaggccatcgtggttatccgggtctggatggtgctaaaggattcccgggaaccccgggcctgccgggcgttaagggtcaccgtggttacccgggcctggatggcgctaagggtttcccgggtacgcccggcctgccgggcgtcaaaggtcatcgtggttacccgggtttagacggcgcaaaaggtttcccgggaaccccgggtctgccgggtgttaagggccatcgtggctatccgggcttggacggtgcaaagggttttcctggtactccaggcttgcccggcgttaagggccaccgtggttacccgggtttggacggcgctaaaggctttccgggaaccccgggtcttccgggcgtgaaaggtcaccgtggttacccgggtctggacggcgcgaag

SEQ ID NO: 25 - DNA, 1008 bp, synthetic construct
  source 1..1008: mol_type = other DNA
ggaacacccgggctgccgggtgttaagggccatcgtggctacccgggtttggacggtgcgaaaggcacccctggcctgccgggtgtcaaaggccatcgtggttatccgggtctcgacggtgcgaagggtaccccaggactgccgggtgttaaaggtcaccgcggttacccgggtctggacggcgcaaaaggtactccaggcctgccgggcgtgaagggtcatcgtggttacccgggcctggacggcgcgaagggcaccccgggcttaccgggcgtgaaaggccatcgtggttatccggggttggatggcgcaaagggtaccccgggtctgcctggtgttaagggccaccgcggttatccgggcctggatggtgcgaaaggtacgccgggattgccgggtgtgaagggtcatcgtggttacccgggtctggatggtgccaaaggcacgccaggccttccgggcgtcaagggccaccgcggttacccgggcctggatggtgcgaaaggtaccccgggtttgcctggtgttaagggccaccgcggttatcctggtttggacggcgcgaaaggaaccccgggcctgccgggtgttaaaggccatcgtggctacccgggtctggacggcgctaaaggcactccgggtctgccgggcgtgaagggccaccgtggttatccgggtttagacggcgcgaaaggcaccccaggcctgccgggtgtcaagggtcaccgcggttacccgggtctggatggtgccaagggcaccccgggcttgccgggcgtgaaaggacatcgtggttacccgggcctggatggtgctaagggcacgccaggtcttccgggtgtgaaaggtcaccgtggttatccgggtctggacggtgcaaagggaaccccggggctgccgggcgtaaaaggccacagaggttatccgggtcttgatggtgcgaagggcaccccgggcctgccgggcgttaaaggtcaccgtggttacccgggtttggacggcgctaaa

SEQ ID NO: 26 - DNA, 936 bp, synthetic construct
  source 1..936: mol_type = other DNA
ggagaaagggggttgaagggacaccgcggttttactggtttgcaaggcctgccgggccctccgggtccgtctggcgatcagggtgcaagcggcccggcgggtccgtcgggcccgcgtggtgagcgcggtcttaagggccatcgtggtttcaccggtttacaaggtctgccgggcccgccgggtccgagcggtgatcaaggggcctccggtccggctggcccgtccggcccaagaggcgaacgtggtctgaaaggtcatcgtggattcaccggactgcagggtctgcctggtccgcctggtccgtcaggcgaccaaggtgcgagcggtccggcgggtccgtccggtccgcgtggtgaacgtggtctgaaaggccaccgcggcttcaccggtttgcaaggcctgccaggcccaccgggtccgtctggcgaccagggagccagcggtccggctggcccatctggcccacgcggcgagcgcggtctgaaaggccaccgtggctttacgggcttgcagggtctcccgggcccaccgggcccgagcggtgatcagggtgccagcggaccggcaggcccctctggtccgcgtggtgaacgtggcctgaaaggtcatcgtggttttaccggtttacagggcctgccaggtcccccgggtccgtccggcgaccagggcgcaagcggtccggctggcccgagcggtccgcgtggcgagcgcggccttaagggccacagaggcttcacgggtctgcaaggtttgccgggtccgcctggcccgtcgggcgatcagggcgcgagcggcccggcgggtccgagcggtccgcgtggcgagcgtggtctgaagggtcaccgcggttttaccggtctgcaaggtctgccgggtccgcctggcccgagcggcgaccagggagcgagcggtccggcgggtccgagtggtccgcgt

SEQ ID NO: 27 - DNA, 990 bp, synthetic construct
  source 1..990: mol_type = other DNA
ggggaaaggggactcaaaggtcaccgcggtttcacgggccttcaaggtctgccgggtcctccgggtccgagcggcgaccaaggtgcgtctggcccagcgggtgagcgtggtttaaaaggccaccgcggtttcaccggcctgcagggtttaccgggtccgcctggcccgagcggtgatcaaggtgcaagcggcccggcaggcgaacgcggtctgaaaggccatagaggttttaccggcctgcagggcttgccgggcccgccgggcccgagtggcgatcaaggtgcttccggcccggcgggtgaacgtggcctgaagggccatcgtggctttaccggtctgcagggcctgccaggtccgccgggcccgtctggcgaccagggtgcgagcggtccagccggtgagcgcggcttgaagggccaccgcggctttacgggtttgcaaggtctgcctggtccgccgggcccgtcaggcgatcaaggggcgagcggcccggcgggtgaacgtggtctgaaaggtcatcgtggattcaccggcctgcagggtctgccgggcccgcccggcccgtccggtgaccagggtgcttccggtccggctggtgagcgcggtcttaagggacaccgtggcttcaccggtctgcagggcttgccgggtcctccggggccgagcggcgaccagggtgcgtccggcccggcgggtgaacgtggtctgaagggccaccgtggttttaccggcttgcaaggtctgccgggtccaccgggtccgtctggcgatcagggagccagcggtccggcaggcgagcgtggtttgaagggtcaccgtggattcaccggcctgcaggggctgccgggcccgccgggtccgtcgggcgatcagggagcgagcggtccggcaggtgagcgtggtctgaaaggccatcgtggcttcactggtttgcaaggcctgcctggcccaccgggtccgagcggtgaccagggtgccagcggtccggct

SEQ ID NO: 28 - DNA, 972 bp, synthetic construct
  source 1..972: mol_type = other DNA
ggagaaagggggcttaagggccatcgtggcttcacgggtttgcagggcctgccgggcccaccgggtccgagcggcgatcaaggcgagcggggcctgaaaggtcatcgtggctttaccggtttgcagggcctgccgggcccaccgggaccgagcggtgatcagggggagcgtggtctgaaaggtcatcgtggttttaccggtctgcagggtttgccgggtcctccgggtccgtctggcgaccaaggtgagcgtggtctgaaaggtcatcgtggtttcaccggtttacaaggcctgccgggcccaccgggtccgagcggtgaccaaggcgagcgtggcctgaaaggccaccgcggtttcaccggtcttcagggtctgccgggcccaccgggtcccagcggtgaccagggtgaacgcggtctgaagggtcacagaggcttcaccggtctccaaggcttaccgggtccgccgggcccgagcggtgatcagggcgaacgtggtctgaagggccaccgtggctttacgggtctgcaaggcctgccgggtccgccgggtccgtcgggcgaccagggtgagcgcggtttgaagggccaccgtggattcaccggcctgcagggcctgccgggaccgcctggtccgtcaggtgatcagggtgagcgcggtctcaagggtcatcgtggttttaccggtttacaaggtttgccgggtccgcctggcccgtctggtgatcaaggcgaacgtggtctgaaaggccaccgcggcttcactggtctgcagggcttgccgggcccaccgggtccgtccggcgatcaaggcgaacgtggtctgaagggtcaccgcggattcacgggcctgcagggcctgccgggtccgccaggtccgtccggcgaccagggcgaacgcgggctgaaaggtcaccgtggctttaccggtttgcaaggactgccgggtccgccgggcccgagcggcgaccag

SEQ ID NO: 29 - DNA, 1008 bp, synthetic construct
  source 1..1008: mol_type = other DNA
ggagaaagggggctgaagggtcaccgtggttttaccggtttgcaaggtttgccgggtccgccgggtgagcgcggcctgaagggtcatcgtggcttcaccggcctgcaaggcctgccgggtccgccgggtgagcgtggtctcaagggtcatcgtggctttaccggtttacagggtctgccgggcccaccgggcgagcgcggtctgaaaggccatcgtggattcaccggcctgcagggcttgccgggtccaccgggcgaaagaggcttaaaaggtcaccgtggttttacgggtctgcaaggtctgccgggtccgccgggtgaacgtggccttaagggtcaccgcggcttcactggtctgcagggtttgccgggtccgcctggtgaaaggggtctgaaaggccatcgtggtttcaccggtctgcagggcctgccgggcccaccgggtgagagaggcttgaagggtcaccgtggttttacgggcctgcagggtctgccgggcccgccgggtgagcgcggtcttaagggccaccgtggattcaccggccttcaaggtctgccgggtccgccgggggagcgtggcctgaaaggtcatcgcggcttcaccggtttgcaaggtttgccaggcccaccgggcgaacgtggcctgaaagggcaccgtggttttactggtttgcagggcctgccgggcccgccgggcgagcgcggtttgaagggccaccgtggtttcacgggcctgcaaggtctgccgggccctccgggagaacgcggtctgaaaggtcaccgtggcttcaccggcctgcagggtctaccgggtccaccgggcgagcgcggactgaaaggtcatcgcggcttcaccggtctgcagggcctgccgggtccgccgggtgaacgtggcctgaaaggccaccgcggttttaccggtttacaaggcttgccgggtccgccgggtgaacgtggcttgaagggccatcgtggctttaccggtcttcaggggctgccgggcccgcct